European Patent Application EP 4 741 416 A1, published May 13, 2026. Title: Method for producing a trypsin-like protease in Bacillus. Applicant: c-LEcta GmbH. Application WO. The sequence listing filed with the application follows.

SEQUENCE LISTING (206 sequences)

SEQ ID NO: 1 - protein, 224 aa, Fusarium oxysporum
IVGGTSASAGDFPFIVSISRNGGPWCGGSLLNANTVLTAAHCVSGYAQSGFQIRAGSLSRTSGGITSSLSSVRVHPSYSGNNNDLAILKLSTSIPSGGNIGYARLAASGSDPVAGSSATVAGWGATSEGGSSTPVNLLKVTVPIVSRATCRAQYGTSAITNQMFCAGVSSGGKDSCQGDSGGPIVDSSNTLIGAVSWGNGCARPNYSGVYASVGALRSFIDTYA

SEQ ID NO: 2 - protein, 7 aa, Fusarium oxysporum
APQEIPN

SEQ ID NO: 3 - protein, 9 aa, synthetic construct
AAAPQEIPN

SEQ ID NO: 4 - protein, 9 aa, synthetic construct
APAPQEIPN

SEQ ID NO: 5 - protein, 9 aa, synthetic construct
AAAPREIPN

SEQ ID NO: 6 - protein, 9 aa, synthetic construct
AAAPQEAPN

SEQ ID NO: 7 - protein, 9 aa, synthetic construct
APAPREAPR

SEQ ID NO: 8 - protein, 9 aa, synthetic construct
AAAPQEIPK

SEQ ID NO: 9 - protein, 9 aa, synthetic construct
AAAPQEIPR

SEQ ID NO: 10 - protein, 9 aa, synthetic construct
AAAPREAPR

SEQ ID NO: 11 - protein, 9 aa, synthetic construct
APAPREAPK

SEQ ID NO: 12 - protein, 9 aa, synthetic construct
APAPQEAPR

SEQ ID NO: 13 - protein, 9 aa, synthetic construct
APAPREIPR

SEQ ID NO: 14 - protein, 7 aa, synthetic construct
APQEIPK

SEQ ID NO: 15 - protein, 7 aa, synthetic construct
APQEIPR

SEQ ID NO: 16 - protein, 9 aa, synthetic construct
APAPQEIPK

SEQ ID NO: 17 - protein, 9 aa, synthetic construct
APAPQEIPR

SEQ ID NO: 18 - protein, 9 aa, synthetic construct
AAAPREIPK

SEQ ID NO: 19 - protein, 9 aa, synthetic construct
AAAPREIPR

SEQ ID NO: 20 - protein, 9 aa, synthetic construct
AAAPQEAPK

SEQ ID NO: 21 - protein, 9 aa, synthetic construct
AAAPQEAPR

SEQ ID NO: 22 - skipped

SEQ ID NO: 23 - protein, 4 aa, synthetic construct
AAPR

SEQ ID NO: 24 - protein, 5 aa, synthetic construct
AAAPR

SEQ ID NO: 25 - protein, 5 aa, synthetic construct
APAPR

SEQ ID NO: 26 - protein, 7 aa, synthetic construct
QPREAPR

SEQ ID NO: 27 - protein, 8 aa, synthetic construct
FPVDDDDR

SEQ ID NO: 28 - protein, 8 aa, Bos taurus
FPVDDDDK

SEQ ID NO: 29 - protein, 10 aa, synthetic construct
AAFPVDDDDR

SEQ ID NO: 30 - protein, 10 aa, synthetic construct
APFPVDDDDR

SEQ ID NO: 31 - protein, 8 aa, synthetic construct
APVDDDDR

SEQ ID NO: 32 - protein, 9 aa, synthetic construct
AAPVDDDDR

SEQ ID NO: 33 - protein, 10 aa, synthetic construct
APAPVDDDDR

SEQ ID NO: 34 - protein, 6 aa, synthetic construct
ADFSAK

SEQ ID NO: 35 - protein, 6 aa, synthetic construct
ADFSAR

SEQ ID NO: 36 - protein, 9 aa, synthetic construct
TRQPREVPR

SEQ ID NO: 37 - protein, 6 aa, synthetic construct
AAVDRR

SEQ ID NO: 38 - protein, 17 aa, Fusarium oxysporum
MVKFASVVALVAPLAAA

SEQ ID NO: 39 - protein, 41 aa, Bacillus subtilis
MKKMSLFQNMKSKLLPIAAVSVLTAGIFAGAELQQTEKASA

SEQ ID NO: 40 - protein, 28 aa, Bacillus subtilis
MKRLFMKASLVLFAVVFVFAVKGAPAKA

SEQ ID NO: 41 - protein, 26 aa, Bacillus subtilis
MKRITINIITMFIAAAVISLTGTAEA

SEQ ID NO: 42 - protein, 25 aa, Bacillus subtilis
MVKKWLIQFAVMLSVLSTFTYSASA

SEQ ID NO: 43 - protein, 28 aa, Bacillus subtilis
MLKKVILAAFILVGSTLGAFSFSSDASA

SEQ ID NO: 44 - protein, 32 aa, Bacillus subtilis
MKKKKTWKRFLHFSSAALAAGLIFTSAAPAEA

SEQ ID NO: 45 - protein, 28 aa, Bacillus subtilis
MKQGKFSVFLILLLMLTLVVAPKEKAEA

SEQ ID NO: 46 - protein, 28 aa, Bacillus subtilis
MKRMIVRMTLPLLIVCLAFSSFSASARA

SEQ ID NO: 47 - protein, 26 aa, Bacillus subtilis
MLTKRLLTIYIMLLGLIAWFPGAAQA

SEQ ID NO: 48 - protein, 23 aa, Bacillus subtilis
MKRLLSTLLIGIMLLTFAPSAFA

SEQ ID NO: 49 - protein, 24 aa, Bacillus subtilis
MRSYIKVLTMCFLGLILFVPTALA

SEQ ID NO: 50 - protein, 47 aa, Bacillus subtilis
MAKPLSKGGILVKKVLIAGAVGTAVLFGTLSSGIPGLPAADAQVAKA

SEQ ID NO: 51 - protein, 26 aa, Bacillus subtilis
MKKGIIRFLLVSFVLFFALTPTGVQA

SEQ ID NO: 52 - protein, 26 aa, Bacillus subtilis
MMKKLFHSTLIVLLFFSFFGVQPIHA

SEQ ID NO: 53 - protein, 24 aa, Bacillus subtilis
LKKIWIGMLAAAVLLLMVPKVSLA

SEQ ID NO: 54 - protein, 28 aa, Bacillus subtilis
MKRKLLSSLAISALSLGLLVSAPTASFA

SEQ ID NO: 55 - protein, 27 aa, Bacillus subtilis
MRKYTVIASILLSFLSVLSGGHHESKA

SEQ ID NO: 56 - protein, 32 aa, Bacillus subtilis
MNTLANWKKFLLVAVIICFLVPIMTKAEIAEA

SEQ ID NO: 57 - protein, 41 aa, Bacillus subtilis
MVKSFRMKALIAGAAVAAAVSAGAVSDVPAAKVLQPTAAYA

SEQ ID NO: 58 - protein, 38 aa, Bacillus amyloliquefaciens
MSLFKQVRSKLLPAAAVSVLTAGLIAGAGLQHSEQAAA

SEQ ID NO: 59 - protein, 28 aa, Bacillus amyloliquefaciens
MKRLFTKASLVLFAVVFVFAVKGAPAKA

SEQ ID NO: 60 - protein, 24 aa, Bacillus amyloliquefaciens
MKKAALSLAAFFITAMVFTMPAHA

SEQ ID NO: 61 - protein, 25 aa, Bacillus amyloliquefaciens
MVKKWLIQFAVMLSVLSTFTYSASA

SEQ ID NO: 62 - protein, 27 aa, Bacillus amyloliquefaciens
MKKLFLALLILAGSTLGAISYSSDASA

SEQ ID NO: 63 - protein, 30 aa, Bacillus amyloliquefaciens
MKNRFKRLIRFSCAAVTAGLLLMSSSPASA

SEQ ID NO: 64 - protein, 29 aa, Bacillus amyloliquefaciens
MKKVSKILMGASALLIAGSTFICSPKAEA

SEQ ID NO: 65 - protein, 25 aa, Bacillus amyloliquefaciens
MHKTRLIVCAVLLIAAAVWMPEAKA

SEQ ID NO: 66 - protein, 23 aa, Bacillus amyloliquefaciens
MKRLISTLLIGILLTASAPSAFA

SEQ ID NO: 67 - protein, 24 aa, Bacillus amyloliquefaciens
MRSYLKVLIISMLGLILFIPSALA

SEQ ID NO: 68 - protein, 22 aa, Bacillus amyloliquefaciens
MMKKGLLAGVLTTAVLFGACTA

SEQ ID NO: 69 - protein, 25 aa, Bacillus amyloliquefaciens
MKKGIIRYLLPAFVLSFTLSTSSQA

SEQ ID NO: 70 - protein, 19 aa, Bacillus amyloliquefaciens
MRKLFHATLILLLSFSFFA

SEQ ID NO: 71 - protein, 26 aa, Bacillus amyloliquefaciens
MKKMWIGLLAAAVVLCTIPKISLADA

SEQ ID NO: 72 - protein, 28 aa, Bacillus amyloliquefaciens
MKHKFFSTVMASLFGLVLLLSLPTASFA

SEQ ID NO: 73 - protein, 22 aa, Bacillus amyloliquefaciens
MKLVMTLFFLIGLLCVSPSADA

SEQ ID NO: 74 - protein, 24 aa, Bacillus amyloliquefaciens
MLTSWRKYILAGLMICLVAPAVTR

SEQ ID NO: 75 - protein, 18 aa, Bacillus amyloliquefaciens
MKTLAAGAAVAAALSVGA

SEQ ID NO: 76 - protein, 29 aa, Bacillus subtilis
MKKKQVMLALTAAAGLGLTALHSAPAAKA

SEQ ID NO: 77 - protein, 35 aa, Bacillus subtilis
MKISMQKADFWKKAAISLLVFTMFFTLMMSETVFA

SEQ ID NO: 78 - protein, 27 aa, Bacillus subtilis
MKKRLIAPMLLSAASLAFFAMSGSAQA

SEQ ID NO: 79 - protein, 30 aa, Bacillus subtilis
MRKKTKNRLISSVLSTVVISSLLFPGAAGA

SEQ ID NO: 80 - protein, 32 aa, Bacillus subtilis
MKKRKRRNFKRFIAAFLVLALMISLVPADVLA

SEQ ID NO: 81 - protein, 29 aa, Bacillus subtilis
MKRSISIFITCLLITLLTMGGMIASPASA

SEQ ID NO: 82 - protein, 25 aa, Bacillus subtilis
MKSCKQLIVCSLAAILLLIPSVSFA

SEQ ID NO: 83 - protein, 31 aa, Bacillus subtilis
MKFVKRRIIALVTILMLSVTSLFALQPSAKA

SEQ ID NO: 84 - protein, 25 aa, Bacillus subtilis
MKIRKILLSSALSFGMLISAVPALA

SEQ ID NO: 85 - protein, 34 aa, Bacillus subtilis
MKKIVAAIVVIGLVFIAFFYLYSRSGDVYQSVDA

SEQ ID NO: 86 - protein, 28 aa, Bacillus subtilis
MPYLKRVLLLLVTGLFMSLFAVTATASA

SEQ ID NO: 87 - protein, 26 aa, Bacillus subtilis
MNFKKTVVSALSISALALSVSGVASA

SEQ ID NO: 88 - protein, 25 aa, Bacillus subtilis
MKTKTLFIFSAILTLSIFAPNETFA

SEQ ID NO: 89 - protein, 26 aa, Bacillus subtilis
MRKNRILALFVLSLGLLSFMVTPVSA

SEQ ID NO: 90 - protein, 24 aa, Bacillus subtilis
MKKRLIQVMIMFTLLLTMAFSADA

SEQ ID NO: 91 - protein, 28 aa, Bacillus subtilis
MTKKAWFLPLVCVLLISGWLAPAASASA

SEQ ID NO: 92 - protein, 32 aa, Bacillus subtilis
MKKFPKKLLPIAVLSSIAFSSLASGSVPEASA

SEQ ID NO: 93 - protein, 27 aa, Bacillus subtilis
MKVFIVIMIIVVIFFALILLDIFMGRA

SEQ ID NO: 94 - protein, 28 aa, Bacillus subtilis
MKKVLMAFIICLSLILSVLAAPPSGAKA

SEQ ID NO: 95 - protein, 26 aa, Bacillus subtilis
MKKSQYFIVFICFFVLFSVHPIAAAA

SEQ ID NO: 96 - protein, 27 aa, Bacillus subtilis
MRIFKKAVFVIMISFLIATVNVNTAHA

SEQ ID NO: 97 - protein, 29 aa, Bacillus subtilis
MNIKKFAKQATVLTFTTALLAGGATQAFA

SEQ ID NO: 98 - protein, 27 aa, Bacillus subtilis
MNKKYFVLIVCIIFTSALFPTFSSVTA

SEQ ID NO: 99 - protein, 31 aa, Bacillus subtilis
MKKTFVKKAMLTTAAMTSAALLTFGPDAASA

SEQ ID NO: 100 - protein, 28 aa, Bacillus subtilis
MFKKLLLATSALTFSLSLVLPLDGHAKA

SEQ ID NO: 101 - protein, 28 aa, Bacillus subtilis
MRNLTKTSLLLAGLCTAAQMVFVTHASA

SEQ ID NO: 102 - protein, 27 aa, Bacillus subtilis
MKKIGLLFMLCLAALFTIGFPAQQADA

SEQ ID NO: 103 - protein, 34 aa, Bacillus subtilis
MKQFAITLSVLCALILLVPTLLVIPFQHNKEAGA

SEQ ID NO: 104 - protein, 23 aa, Bacillus subtilis
MKKRFSLIMMTGLLFGLTSPAFA

SEQ ID NO: 105 - protein, 27 aa, Bacillus subtilis
MKKWLIIAVSLAIAIVLFMYTKGEAKA

SEQ ID NO: 106 - protein, 28 aa, Bacillus subtilis
MFKFKKNFLVGLSAALMSISLFSATASA

SEQ ID NO: 107 - protein, 23 aa, Bacillus subtilis
MRKTIFAFLTGLMMFGTITAASA

SEQ ID NO: 108 - protein, 21 aa, Bacillus subtilis
MTTKFTALAVFLLCFMPAAKI

SEQ ID NO: 109 - protein, 27 aa, Bacillus subtilis
MGLGKKLSVAVAASFMSLSISLPGVQA

SEQ ID NO: 110 - protein, 25 aa, Bacillus subtilis
MKKRLIGFLVLVPALIMSGITLIEA

SEQ ID NO: 111 - protein, 22 aa, Bacillus subtilis
MMIKQCVICLSLLVFGTTAAHA

SEQ ID NO: 112 - protein, 30 aa, Bacillus subtilis
MRKSLITLGLASVIGTSSFLIPFTSKTASA

SEQ ID NO: 113 - protein, 26 aa, Bacillus subtilis
MKKAFILSAAAAVGLFTFGGVQQASA

SEQ ID NO: 114 - protein, 43 aa, Bacillus subtilis
MFRLFHNQQKAKTKLKVLLIFQLSVIFSLTAAICLQFSDDTSA

SEQ ID NO: 115 - protein, 34 aa, Bacillus subtilis
MKLVPRFRKQWFAYLTVLCLALAAAVSFGVPAKA

SEQ ID NO: 116 - protein, 27 aa, Bacillus subtilis
MGMKKKLSLGVASAALGLALVGGGTWA

SEQ ID NO: 117 - protein, 23 aa, Bacillus subtilis
MKKLLAAGIIGLLTVSIASPSFA

SEQ ID NO: 118 - protein, 26 aa, Bacillus subtilis
MKKKLAAGLTASAIVGTTLVVTPAEA

SEQ ID NO: 119 - protein, 26 aa, Bacillus subtilis
MAAQTDYKKQVVGILLSLAFVLFVFS

SEQ ID NO: 120 - protein, 26 aa, Bacillus subtilis
MTMLRKIIGWILLLCIIPLFAFTVIA

SEQ ID NO: 121 - protein, 24 aa, Bacillus subtilis
MKRLCLWFTVFSLFLVLLPGKALG

SEQ ID NO: 122 - protein, 40 aa, Bacillus subtilis
MREEEKKTSQVKKLQQFFRKRWVFPAIYLVSAAVILTAVL

SEQ ID NO: 123 - protein, 27 aa, Bacillus subtilis
MKWNPLIPFLLIAVLGIGLTFFLSVKG

SEQ ID NO: 124 - protein, 32 aa, Bacillus subtilis
MGNTRKKVSVIGAGFTGATTAFLIAQKELADV

SEQ ID NO: 125 - protein, 22 aa, Bacillus subtilis
MKLAKRVSALTPSTTLAITAKA

SEQ ID NO: 126 - protein, 35 aa, Bacillus subtilis
MLRKKHFSWMLVILILIAVLSFIKLPYYITKPGEA

SEQ ID NO: 127 - protein, 23 aa, Bacillus subtilis
MKRFILVLSFLSIIVAYPIQTNA

SEQ ID NO: 128 - protein, 26 aa, Bacillus subtilis
MKLSVKIAGVLTVAAAAMTAKMYATA

SEQ ID NO: 129 - protein, 23 aa, Bacillus subtilis
MNNNKLLLVDGMALLFRAFFATA

SEQ ID NO: 130 - protein, 38 aa, Bacillus subtilis
MGRIKTKITILLVLLLLLAGGYMYINDIELKDVPTAIG

SEQ ID NO: 131 - protein, 25 aa, Bacillus subtilis
MKTLRTLCVLMILSGVIFFGLKIDA

SEQ ID NO: 132 - protein, 28 aa, Bacillus subtilis
MKRLLVSLRVWMVFLMNWVTPDRKTAAA

SEQ ID NO: 133 - protein, 30 aa, Bacillus subtilis
MLKRTSFVSSLFISSAVLLSILLPSGQAHA

SEQ ID NO: 134 - protein, 24 aa, Bacillus subtilis
MKMKSGMEQAVSVLLLLSRLPVQA

SEQ ID NO: 135 - protein, 28 aa, Bacillus subtilis
MKKKQVSHAIIISVMLSFVIAVFHTIHA

SEQ ID NO: 136 - protein, 27 aa, Bacillus subtilis
MRKWYFILLAGVLTSVILAFVYDKTKA

SEQ ID NO: 137 - protein, 30 aa, Bacillus subtilis
MNKPTKLFSTLALAAGMTAAAAGGAGTIHA

SEQ ID NO: 138 - protein, 39 aa, Bacillus subtilis
MEERSQRRKKKRKLKKWVKVVAGLMAFLVIAAGSVGAYA

SEQ ID NO: 139 - protein, 21 aa, Bacillus subtilis
MKKVMLATALFLGLTPAGANA

SEQ ID NO: 140 - protein, 36 aa, Bacillus subtilis
MKLKTKASIKFGICVGLLCLSITGFTPFFNSTHAEA

SEQ ID NO: 141 - protein, 35 aa, Bacillus subtilis
MRIQKRRTHVENILRILLPPIMILSLILPTPPIHA

SEQ ID NO: 142 - protein, 30 aa, Bacillus subtilis
MKVCQKSIVRFLVSLIIGTFVISVPFMANA

SEQ ID NO: 143 - protein, 30 aa, Bacillus subtilis
MGESTSLKEILSTLTKRILLIMIVTAAATA

SEQ ID NO: 144 - protein, 26 aa, Bacillus subtilis
MRKKITLACKTCGNRNYTTMKSSASA

SEQ ID NO: 145 - protein, 26 aa, Bacillus subtilis
MKKKIVAGLAVSAVVGSSMAAAPAEA

SEQ ID NO: 146 - protein, 21 aa, Bacillus subtilis
MKKLVLCVSILAVILSGVALT

SEQ ID NO: 147 - protein, 29 aa, Bacillus subtilis
MKLKSKLFVICLAAAAIFTAAGVSANAEA

SEQ ID NO: 148 - protein, 28 aa, Bacillus subtilis
MKKRITYSLLALLAVVAFAFTDSSKAKA

SEQ ID NO: 149 - protein, 24 aa, Bacillus subtilis
MKKMLMLAFTFLLALTIHVGEASA

SEQ ID NO: 150 - protein, 33 aa, Bacillus subtilis
MYKKFVPFAVFLFLFFVSFEMMENPHALDYIGA

SEQ ID NO: 151 - protein, 29 aa, Bacillus subtilis
MKSKGSIMACLILFSFTITTFINTETISA

SEQ ID NO: 152 - protein, 32 aa, Bacillus subtilis
MKWNNMLKAAGIAVLLFSVFAYAAPSLKAVQA

SEQ ID NO: 153 - protein, 29 aa, Bacillus subtilis
MKKWMAGLFLAAAVLLCLMVPQQIQGASS

SEQ ID NO: 154 - protein, 24 aa, Bacillus subtilis
MKKLLTVMTMAVLTAGTLLLPAQS

SEQ ID NO: 155 - protein, 29 aa, Bacillus subtilis
MKLWMRKTLVVLFTIVTFGLVSPPAALMA

SEQ ID NO: 156 - protein, 31 aa, Bacillus subtilis
MKRRKFSSVVAAVLIFALIFSLFSPGTKAAA

SEQ ID NO: 157 - protein, 26 aa, Bacillus subtilis
MKKELLASLVLCLSLSPLVSTNEVFA

SEQ ID NO: 158 - protein, 40 aa, Bacillus subtilis
MARKKKKKHEDEHVDESWLVPYADILTLLLALFIVLYASS

SEQ ID NO: 159 - protein, 26 aa, Bacillus subtilis
MFKKHTISLLIIFLLASAVLAKPIEA

SEQ ID NO: 160 - protein, 25 aa, Bacillus subtilis
MKKQIITATTAVVLGSTLFAGAASA

SEQ ID NO: 161 - protein, 26 aa, Bacillus subtilis
MKLKSKLLLSCLALSTVFVATTIANA

SEQ ID NO: 162 - protein, 34 aa, Bacillus subtilis
LRGKSAVLLSLIMLIAGFLISFSFQMTKENNKSA

SEQ ID NO: 163 - protein, 21 aa, Bacillus subtilis
MKLERLLAMVVLLISKKQVQA

SEQ ID NO: 164 - protein, 25 aa, Bacillus subtilis
MKKTIMSFVAVAALSTTAFGAHASA

SEQ ID NO: 165 - protein, 26 aa, Bacillus subtilis
MKVPKTMLLSTAAGLLLSLTATSVSA

SEQ ID NO: 166 - protein, 25 aa, Bacillus subtilis
MKLRKVLTGSVLSLGLLVSASPAFA

SEQ ID NO: 167 - protein, 28 aa, Bacillus subtilis
MTLTKLKMLSMLTVMIASLFIFSSQALA

SEQ ID NO: 168 - protein, 29 aa, Bacillus subtilis
MHLIRAAGAVCLAVVLIAGCRFNEDQHQA

SEQ ID NO: 169 - protein, 26 aa, Bacillus subtilis
MKRIRIPMTLALGAALTIAPLSFASA

SEQ ID NO: 170 - protein, 26 aa, Bacillus subtilis
MFNRLFRVCFLAALIMAFTLPNSVYA

SEQ ID NO: 171 - protein, 27 aa, Bacillus subtilis
MRKKLKWLSFLLGFIILLFLFKYQFSN

SEQ ID NO: 172 - protein, 21 aa, Bacillus subtilis
MKKRFFGPIILAFILFAGAIA

SEQ ID NO: 173 - protein, 36 aa, Bacillus subtilis
MKKKLMIILLIILIVIGALGAAAYFVLGGKSEKSEA

SEQ ID NO: 174 - protein, 31 aa, Bacillus subtilis
MRNERRKKKKTLLLTILTIIGLLVLGTGGYA

SEQ ID NO: 175 - protein, 23 aa, Bacillus subtilis
MPNKRLMLLLLCIIILVAMIGFS

SEQ ID NO: 176 - protein, 34 aa, Bacillus subtilis
MIQMPKKNKFMNRGAAILSICFALFFFVILGRMA

SEQ ID NO: 177 - protein, 21 aa, Bacillus subtilis
MRNKRRNRQIVVAVNGGKAVK

SEQ ID NO: 178 - protein, 23 aa, Bacillus subtilis
MKKTVIICIYIFLLLSGALVGLA

SEQ ID NO: 179 - protein, 28 aa, Bacillus subtilis
MKISKRMKLAVIAFLIVFFLLLLRLAEI

SEQ ID NO: 180 - protein, 36 aa, Bacillus subtilis
MSNNQSRYENRDKRRKANLVLNILIAIVSILIVVVA

SEQ ID NO: 181 - protein, 25 aa, Bacillus subtilis
MNYIKAGKWLTVFLTFLGILLFIDL

SEQ ID NO: 182 - protein, 19 aa, Bacillus subtilis
MKVLLSALLLLLFAFEPSA

SEQ ID NO: 183 - protein, 25 aa, Bacillus subtilis
MKTLWKVLKIVFVSLAALVLLVSVS

SEQ ID NO: 184 - protein, 41 aa, Bacillus subtilis
MTSPTRRRTAKRRRRKLNKRGKLLFGLLAVMVCITIWNALH

SEQ ID NO: 185 - protein, 28 aa, Bacillus subtilis
MRKKRVITCVMAASLTLGSLLPAGYASA

SEQ ID NO: 186 - protein, 34 aa, Bacillus subtilis
MKKKTKIILSLLAALIVILIVLPVLSPVVFTASS

SEQ ID NO: 187 - protein, 27 aa, Bacillus subtilis
MKKWIVLFLVLIAAAISIFVYVSTGSE

SEQ ID NO: 188 - protein, 34 aa, Bacillus subtilis
MTKRGIQAFAGGIILATAVLAAVFYLTDEDQAAA

SEQ ID NO: 189 - protein, 37 aa, Bacillus subtilis
MSGKKKESGKFRSVLLIIILPLMFLLIAGGIVLWAAG

SEQ ID NO: 190 - protein, 25 aa, Bacillus subtilis
MRFTKVVGFLSVLGLAAVFPLTAQA

SEQ ID NO: 191 - protein, 26 aa, Bacillus subtilis
MLKKKWMVGLLAGCLAAGGFSYNAFA

SEQ ID NO: 192 - protein, 33 aa, Bacillus subtilis
MKLFNRKVTLVSLILMAVFQFFMALIIKRIVIS

SEQ ID NO: 193 - protein, 30 aa, Bacillus subtilis
MDKFLNNRWAVKIIALLFALLLYVAVNSNQ

SEQ ID NO: 194 - protein, 33 aa, Bacillus subtilis
MKKVWIGIGIAVIVALFVGINIYRSAAPTSGSA

SEQ ID NO: 195 - protein, 28 aa, Bacillus subtilis
MELSFTKILVILFVGFLVFGPDKLPALG

SEQ ID NO: 196 - protein, 35 aa, Bacillus subtilis
MNKWKRLFFILLAINFILAAGFVALVLLPGEQAQV

SEQ ID NO: 197 - protein, 36 aa, Bacillus subtilis
MKKKQQSSAKFAVILTVVVVVLLAAIVIINNKTEQG

SEQ ID NO: 198 - protein, 33 aa, Bacillus subtilis
MFAKRFKTSLLPLFAGFLLLFHLVLAGPAAASA

SEQ ID NO: 199 - protein, 30 aa, Bacillus subtilis
MNKFLKSNFRFLLAAALGISLLASSNFIKA

SEQ ID NO: 200 - protein, 25 aa, Bacillus subtilis
MKGNIYSLFVLIAAFFWGTTGTVQA

SEQ ID NO: 201 - protein, 21 aa, Bacillus subtilis
MKSLPYTIALLFCGLIIVSMA

SEQ ID NO: 202 - protein, 21 aa, Bacillus subtilis
MKKLIMALVILGALGTSYISA

SEQ ID NO: 203 - protein, 27 aa, Bacillus subtilis
MKKAAAVLLSLGLVFGFSYGAGHVAEA

SEQ ID NO: 204 - protein, 21 aa, Bacillus subtilis
MKRFLIGAGVAAVILSGWFIA

SEQ ID NO: 205 - protein, 27 aa, Bacillus subtilis
MKKIVSILFMFGLVMGFSQFQPSTVFA

SEQ ID NO: 206 - protein, 25 aa, Bacillus subtilis
MKSKWMSGLLLVAVGFSFTQVMVHA